European Patent Specification EP 3 968 023 B1, published October 8, 2025. Title: ASSAYS FOR SINGLE MOLECULE DETECTION AND USE THEREOF. Applicant: SINGULAR BIO, INC. FEHR, Adrian Nielsen COLLINS, Patrick James HERSCHLEB, Jill Lyndon JONES, Hywel Bowden. The sequence listing filed with the application follows.

SEQUENCE LISTING (369 sequences)

SEQ ID NO: 1 - DNA, 60 bp, Artificial Sequence
  Synthetic sequence
gccctcatcttcttccctgcgttctcaccaccctcaccaaggaagaagtgagggcttctc

SEQ ID NO: 2 - DNA, 60 bp, Artificial Sequence
  Synthetic sequence
gccctcatcttcttccctgcgttctcaccaccctcaccaaaaatcaaggtgaccagctcc

SEQ ID NO: 3 - DNA, 62 bp, Artificial Sequence
  Synthetic sequence
gccctcatcttcttccctgcgttctcaccaccctcaccaatcatctgccaagacagaagttc

SEQ ID NO: 4 - DNA, 60 bp, Artificial Sequence
  Synthetic sequence
gccctcatcttcttccctgcgttctcaccaccctcaccaagcaggagagtcaaaggtctg

SEQ ID NO: 5 - DNA, 60 bp, Artificial Sequence
  Synthetic sequence
gccctcatcttcttccctgcgttctcaccaccctcaccaagttgccatggagattgttgc

SEQ ID NO: 6 - DNA, 60 bp, Artificial Sequence
  Synthetic sequence
gccctcatcttcttccctgcgttctcaccaccctcaccaacagctcagtgatgtcattgc

SEQ ID NO: 7 - DNA, 61 bp, Artificial Sequence
  Synthetic sequence
gccctcatcttcttccctgcgttctcaccaccctcaccaaccttgacctctgctaatgtgg

SEQ ID NO: 8 - DNA, 60 bp, Artificial Sequence
  Synthetic sequence
gccctcatcttcttccctgcgttctcaccaccctcaccaacacctgtccaacagctacag

SEQ ID NO: 9 - DNA, 61 bp, Artificial Sequence
  Synthetic sequence
gccctcatcttcttccctgcgttctcaccaccctcaccaaagaatgtatcttcaggcctgc

SEQ ID NO: 10 - DNA, 60 bp, Artificial Sequence
  Synthetic sequence
gccctcatcttcttccctgcgttctcaccaccctcaccaaaagtaatcactctgggtggc

SEQ ID NO: 11 - DNA, 60 bp, Artificial Sequence
  Synthetic sequence
gccctcatcttcttccctgcgttctcaccaccctcaccaaagctcacagacaaccttgtg

SEQ ID NO: 12 - DNA, 60 bp, Artificial Sequence
  Synthetic sequence
gccctcatcttcttccctgcgttctcaccaccctcaccaagcaatagacacctacaggcg

SEQ ID NO: 13 - DNA, 60 bp, Artificial Sequence
  Synthetic sequence
gccctcatcttcttccctgcgttctcaccaccctcaccaagcacattatcaaaggccacg

SEQ ID NO: 14 - DNA, 60 bp, Artificial Sequence
  Synthetic sequence
gccctcatcttcttccctgcgttctcaccaccctcaccaacaacgacctaaagcatgtgc

SEQ ID NO: 15 - DNA, 60 bp, Artificial Sequence
  Synthetic sequence
gccctcatcttcttccctgcgttctcaccaccctcaccaagacatacatggctttggcag

SEQ ID NO: 16 - DNA, 62 bp, Artificial Sequence
  Synthetic sequence
gccctcatcttcttccctgcgttctcaccaccctcaccaagagatactgccacttatgcacg

SEQ ID NO: 17 - DNA, 40 bp, Artificial Sequence
  Synthetic sequence
cgtgctaatagtctcagggcttcctccaccgaacgtgtct

SEQ ID NO: 18 - DNA, 40 bp, Artificial Sequence
  Synthetic sequence
cgacgcttcattgcttcattttcctccaccgaacgtgtct

SEQ ID NO: 19 - DNA, 40 bp, Artificial Sequence
  Synthetic sequence
cttgcgccaaacaattgtccttcctccaccgaacgtgtct

SEQ ID NO: 20 - DNA, 40 bp, Artificial Sequence
  Synthetic sequence
gctgcagagtttgcattcatttcctccaccgaacgtgtct

SEQ ID NO: 21 - DNA, 41 bp, Artificial Sequence
  Synthetic sequence
catacacacagaccgagagtcttcctccaccgaacgtgtct

SEQ ID NO: 22 - DNA, 40 bp, Artificial Sequence
  Synthetic sequence
ggatgtcagccagcataagtttcctccaccgaacgtgtct

SEQ ID NO: 23 - DNA, 40 bp, Artificial Sequence
  Synthetic sequence
gcaagtgccaaacagttctcttcctccaccgaacgtgtct

SEQ ID NO: 24 - DNA, 41 bp, Artificial Sequence
  Synthetic sequence
gattccagcacacttgagtctttcctccaccgaacgtgtct

SEQ ID NO: 25 - DNA, 40 bp, Artificial Sequence
  Synthetic sequence
ccgttgcaggtttaaatggcgccctattgcaagccctctt

SEQ ID NO: 26 - DNA, 40 bp, Artificial Sequence
  Synthetic sequence
caagagtgctttatgggcctgccctattgcaagccctctt

SEQ ID NO: 27 - DNA, 41 bp, Artificial Sequence
  Synthetic sequence
gcactcaaggagatcagactggccctattgcaagccctctt

SEQ ID NO: 28 - DNA, 41 bp, Artificial Sequence
  Synthetic sequence
ggctatcgaactacaaccacagccctattgcaagccctctt

SEQ ID NO: 29 - DNA, 41 bp, Artificial Sequence
  Synthetic sequence
gtagctgtctgtggtgtgatcgccctattgcaagccctctt

SEQ ID NO: 30 - DNA, 42 bp, Artificial Sequence
  Synthetic sequence
caagaaacttcgagccttagcagccctattgcaagccctctt

SEQ ID NO: 31 - DNA, 40 bp, Artificial Sequence
  Synthetic sequence
gtgaaccagtccgagtgaaagccctattgcaagccctctt

SEQ ID NO: 32 - DNA, 41 bp, Artificial Sequence
  Synthetic sequence
gcaaatgatgttcagcaccacgccctattgcaagccctctt

SEQ ID NO: 33 - DNA, 20 bp, Artificial Sequence
  Synthetic sequence
gccctcatcttcttccctgc

SEQ ID NO: 34 - DNA, 20 bp, Artificial Sequence
  Synthetic sequence
gttctcaccaccctcaccaa

SEQ ID NO: 35 - DNA, 20 bp, Artificial Sequence
  Synthetic sequence
ggaagaagtgagggcttctc

SEQ ID NO: 36 - DNA, 20 bp, Artificial Sequence
  Synthetic sequence
aaatcaaggtgaccagctcc

SEQ ID NO: 37 - DNA, 22 bp, Artificial Sequence
  Synthetic sequence
tcatctgccaagacagaagttc

SEQ ID NO: 38 - DNA, 20 bp, Artificial Sequence
  Synthetic sequence
gcaggagagtcaaaggtctg

SEQ ID NO: 39 - DNA, 20 bp, Artificial Sequence
  Synthetic sequence
gttgccatggagattgttgc

SEQ ID NO: 40 - DNA, 20 bp, Artificial Sequence
  Synthetic sequence
cagctcagtgatgtcattgc

SEQ ID NO: 41 - DNA, 21 bp, Artificial Sequence
  Synthetic sequence
ccttgacctctgctaatgtgg

SEQ ID NO: 42 - DNA, 20 bp, Artificial Sequence
  Synthetic sequence
cacctgtccaacagctacag

SEQ ID NO: 43 - DNA, 21 bp, Artificial Sequence
  Synthetic sequence
agaatgtatcttcaggcctgc

SEQ ID NO: 44 - DNA, 20 bp, Artificial Sequence
  Synthetic sequence
aagtaatcactctgggtggc

SEQ ID NO: 45 - DNA, 20 bp, Artificial Sequence
  Synthetic sequence
agctcacagacaaccttgtg

SEQ ID NO: 46 - DNA, 20 bp, Artificial Sequence
  Synthetic sequence
gcaatagacacctacaggcg

SEQ ID NO: 47 - DNA, 20 bp, Artificial Sequence
  Synthetic sequence
gcacattatcaaaggccacg

SEQ ID NO: 48 - DNA, 20 bp, Artificial Sequence
  Synthetic sequence
caacgacctaaagcatgtgc

SEQ ID NO: 49 - DNA, 20 bp, Artificial Sequence
  Synthetic sequence
gacatacatggctttggcag

SEQ ID NO: 50 - DNA, 22 bp, Artificial Sequence
  Synthetic sequence
gagatactgccacttatgcacg

SEQ ID NO: 51 - DNA, 20 bp, Artificial Sequence
  Synthetic sequence
cgtgctaatagtctcagggc

SEQ ID NO: 52 - DNA, 20 bp, Artificial Sequence
  Synthetic sequence
cgacgcttcattgcttcatt

SEQ ID NO: 53 - DNA, 20 bp, Artificial Sequence
  Synthetic sequence
cttgcgccaaacaattgtcc

SEQ ID NO: 54 - DNA, 20 bp, Artificial Sequence
  Synthetic sequence
gctgcagagtttgcattcat

SEQ ID NO: 55 - DNA, 21 bp, Artificial Sequence
  Synthetic sequence
catacacacagaccgagagtc

SEQ ID NO: 56 - DNA, 20 bp, Artificial Sequence
  Synthetic sequence
ggatgtcagccagcataagt

SEQ ID NO: 57 - DNA, 20 bp, Artificial Sequence
  Synthetic sequence
gcaagtgccaaacagttctc

SEQ ID NO: 58 - DNA, 21 bp, Artificial Sequence
  Synthetic sequence
gattccagcacacttgagtct

SEQ ID NO: 59 - DNA, 20 bp, Artificial Sequence
  Synthetic sequence
ccgttgcaggtttaaatggc

SEQ ID NO: 60 - DNA, 20 bp, Artificial Sequence
  Synthetic sequence
caagagtgctttatgggcct

SEQ ID NO: 61 - DNA, 21 bp, Artificial Sequence
  Synthetic sequence
gcactcaaggagatcagactg

SEQ ID NO: 62 - DNA, 21 bp, Artificial Sequence
  Synthetic sequence
ggctatcgaactacaaccaca

SEQ ID NO: 63 - DNA, 21 bp, Artificial Sequence
  Synthetic sequence
gtagctgtctgtggtgtgatc

SEQ ID NO: 64 - DNA, 22 bp, Artificial Sequence
  Synthetic sequence
caagaaacttcgagccttagca

SEQ ID NO: 65 - DNA, 20 bp, Artificial Sequence
  Synthetic sequence
gtgaaccagtccgagtgaaa

SEQ ID NO: 66 - DNA, 21 bp, Artificial Sequence
  Synthetic sequence
gcaaatgatgttcagcaccac

SEQ ID NO: 67 - DNA, 20 bp, Artificial Sequence
  Synthetic sequence
ttcctccaccgaacgtgtct

SEQ ID NO: 68 - DNA, 20 bp, Artificial Sequence
  Synthetic sequence
gccctattgcaagccctctt

SEQ ID NO: 69 - DNA, 40 bp, Artificial Sequence
  Synthetic sequence
ttcctccaccgaacgtgtctagaccagcacaacttactcg

SEQ ID NO: 70 - DNA, 37 bp, Artificial Sequence
  Synthetic sequence
ttcctccaccgaacgtgtctccaaatgcacctgcctg

SEQ ID NO: 71 - DNA, 41 bp, Artificial Sequence
  Synthetic sequence
ttcctccaccgaacgtgtctagtttggacaaaggcaattcg

SEQ ID NO: 72 - DNA, 44 bp, Artificial Sequence
  Synthetic sequence
ttcctccaccgaacgtgtcttgagcttagccaatatcaagaagg

SEQ ID NO: 73 - DNA, 42 bp, Artificial Sequence
  Synthetic sequence
ttcctccaccgaacgtgtctacgtgaactttccttggtacac

SEQ ID NO: 74 - DNA, 44 bp, Artificial Sequence
  Synthetic sequence
ttcctccaccgaacgtgtcttgaagatgttctaataccttgccg

SEQ ID NO: 75 - DNA, 38 bp, Artificial Sequence
  Synthetic sequence
ttcctccaccgaacgtgtctcagtgtggagactgaacg

SEQ ID NO: 76 - DNA, 43 bp, Artificial Sequence
  Synthetic sequence
ttcctccaccgaacgtgtctaggcagggtaatgtcatgaaatg

SEQ ID NO: 77 - DNA, 37 bp, Artificial Sequence
  Synthetic sequence
ttcctccaccgaacgtgtctgattgtctggagcgctg

SEQ ID NO: 78 - DNA, 36 bp, Artificial Sequence
  Synthetic sequence
ttcctccaccgaacgtgtctagggagcaataggccg

SEQ ID NO: 79 - DNA, 37 bp, Artificial Sequence
  Synthetic sequence
ttcctccaccgaacgtgtctctgcagggtacaacacg

SEQ ID NO: 80 - DNA, 38 bp, Artificial Sequence
  Synthetic sequence
ttcctccaccgaacgtgtctcgtatctgggaagacggc

SEQ ID NO: 81 - DNA, 40 bp, Artificial Sequence
  Synthetic sequence
ttcctccaccgaacgtgtctcctgtaatcccttgcaatgc

SEQ ID NO: 82 - DNA, 38 bp, Artificial Sequence
  Synthetic sequence
ttcctccaccgaacgtgtctggtctcagcacggttctg

SEQ ID NO: 83 - DNA, 37 bp, Artificial Sequence
  Synthetic sequence
ttcctccaccgaacgtgtctgcacctccctaccacac

SEQ ID NO: 84 - DNA, 41 bp, Artificial Sequence
  Synthetic sequence
ttcctccaccgaacgtgtctgcctctagctagagagaagtc

SEQ ID NO: 85 - DNA, 39 bp, Artificial Sequence
  Synthetic sequence
ttcctccaccgaacgtgtctctggcagtctagccgttac

SEQ ID NO: 86 - DNA, 43 bp, Artificial Sequence
  Synthetic sequence
ttcctccaccgaacgtgtcttgtcttagaatttggcaactggc

SEQ ID NO: 87 - DNA, 39 bp, Artificial Sequence
  Synthetic sequence
ttcctccaccgaacgtgtctgcaggaaagcctactgaac

SEQ ID NO: 88 - DNA, 39 bp, Artificial Sequence
  Synthetic sequence
ttcctccaccgaacgtgtctgggagccagagaaatgtcc

SEQ ID NO: 89 - DNA, 44 bp, Artificial Sequence
  Synthetic sequence
ttcctccaccgaacgtgtcttgtctccagttccacttcatttag

SEQ ID NO: 90 - DNA, 39 bp, Artificial Sequence
  Synthetic sequence
ttcctccaccgaacgtgtctcccgttaattgcctactcg

SEQ ID NO: 91 - DNA, 38 bp, Artificial Sequence
  Synthetic sequence
ttcctccaccgaacgtgtctctcggtcccactggaaag

SEQ ID NO: 92 - DNA, 41 bp, Artificial Sequence
  Synthetic sequence
ttcctccaccgaacgtgtctacacccatgattcagttactg

SEQ ID NO: 93 - DNA, 41 bp, Artificial Sequence
  Synthetic sequence
ttcctccaccgaacgtgtctgctagtatgaacatcacaggc

SEQ ID NO: 94 - DNA, 43 bp, Artificial Sequence
  Synthetic sequence
ttcctccaccgaacgtgtctacaaatgagtaagaagcgagtcg

SEQ ID NO: 95 - DNA, 38 bp, Artificial Sequence
  Synthetic sequence
ttcctccaccgaacgtgtctgataagggttgctctgcg

SEQ ID NO: 96 - DNA, 37 bp, Artificial Sequence
  Synthetic sequence
ttcctccaccgaacgtgtctccatgcaccagctaccc

SEQ ID NO: 97 - DNA, 40 bp, Artificial Sequence
  Synthetic sequence
ttcctccaccgaacgtgtctaactgtaccctactcccagc

SEQ ID NO: 98 - DNA, 41 bp, Artificial Sequence
  Synthetic sequence
ttcctccaccgaacgtgtctaggaccaagggaccagtttag

SEQ ID NO: 99 - DNA, 42 bp, Artificial Sequence
  Synthetic sequence
ttcctccaccgaacgtgtctagagttcctccaagaaattgcg

SEQ ID NO: 100 - DNA, 44 bp, Artificial Sequence
  Synthetic sequence
ttcctccaccgaacgtgtctacattatacagcatgctggctatc

SEQ ID NO: 101 - DNA, 41 bp, Artificial Sequence
  Synthetic sequence
ttcctccaccgaacgtgtctgaggaagaaagtgaggtttgc

SEQ ID NO: 102 - DNA, 44 bp, Artificial Sequence
  Synthetic sequence
ttcctccaccgaacgtgtctctgaattatgtgcttaccaagagc

SEQ ID NO: 103 - DNA, 44 bp, Artificial Sequence
  Synthetic sequence
ttcctccaccgaacgtgtcttgggttctgataaccttatcaagc

SEQ ID NO: 104 - DNA, 39 bp, Artificial Sequence
  Synthetic sequence
ttcctccaccgaacgtgtctggttagtcaaacatgctgc

SEQ ID NO: 105 - DNA, 42 bp, Artificial Sequence
  Synthetic sequence
ttcctccaccgaacgtgtctgacactggcagaatcaaatcac

SEQ ID NO: 106 - DNA, 44 bp, Artificial Sequence
  Synthetic sequence
ttcctccaccgaacgtgtctagagttacacctttagctaaccac

SEQ ID NO: 107 - DNA, 38 bp, Artificial Sequence
  Synthetic sequence
ttcctccaccgaacgtgtctccaggagttcaagaagcg

SEQ ID NO: 108 - DNA, 41 bp, Artificial Sequence
  Synthetic sequence
ttcctccaccgaacgtgtctaccactcctttctcccatctc

SEQ ID NO: 109 - DNA, 44 bp, Artificial Sequence
  Synthetic sequence
ttcctccaccgaacgtgtctgtcttatgggacaatggttgatag

SEQ ID NO: 110 - DNA, 38 bp, Artificial Sequence
  Synthetic sequence
ttcctccaccgaacgtgtctctaccctcaaccctcgtc

SEQ ID NO: 111 - DNA, 38 bp, Artificial Sequence
  Synthetic sequence
ttcctccaccgaacgtgtctccaagactgatcatgccg

SEQ ID NO: 112 - DNA, 40 bp, Artificial Sequence
  Synthetic sequence
gccctattgcaagccctcttagaccagcacaacttactta

SEQ ID NO: 113 - DNA, 37 bp, Artificial Sequence
  Synthetic sequence
gccctattgcaagccctcttccaaattcacctgccca

SEQ ID NO: 114 - DNA, 41 bp, Artificial Sequence
  Synthetic sequence
gccctattgcaagccctcttagtttggacaaaggcgattta

SEQ ID NO: 115 - DNA, 44 bp, Artificial Sequence
  Synthetic sequence
gccctattgcaagccctctttgagcttagccaatatcaacaaga

SEQ ID NO: 116 - DNA, 42 bp, Artificial Sequence
  Synthetic sequence
gccctattgcaagccctcttacgtgaactttccttggtaaat

SEQ ID NO: 117 - DNA, 44 bp, Artificial Sequence
  Synthetic sequence
gccctattgcaagccctctttgaagatgttctaataccttgcta

SEQ ID NO: 118 - DNA, 38 bp, Artificial Sequence
  Synthetic sequence
gccctattgcaagccctcttcagtgtggagaccgaaca

SEQ ID NO: 119 - DNA, 43 bp, Artificial Sequence
  Synthetic sequence
gccctattgcaagccctcttaggcagggtaatgtcatgaagtt

SEQ ID NO: 120 - DNA, 37 bp, Artificial Sequence
  Synthetic sequence
gccctattgcaagccctcttgattgtctggagggctc

SEQ ID NO: 121 - DNA, 36 bp, Artificial Sequence
  Synthetic sequence
gccctattgcaagccctcttagggagcaataggcta

SEQ ID NO: 122 - DNA, 37 bp, Artificial Sequence
  Synthetic sequence
gccctattgcaagccctcttctgcagggtacaagaca

SEQ ID NO: 123 - DNA, 38 bp, Artificial Sequence
  Synthetic sequence
gccctattgcaagccctcttcgtatctgggaagatggg

SEQ ID NO: 124 - DNA, 40 bp, Artificial Sequence
  Synthetic sequence
gccctattgcaagccctcttcctgtaatcccttgcaataa

SEQ ID NO: 125 - DNA, 38 bp, Artificial Sequence
  Synthetic sequence
gccctattgcaagccctcttggtctcagcacggtcctt

SEQ ID NO: 126 - DNA, 37 bp, Artificial Sequence
  Synthetic sequence
gccctattgcaagccctcttgcacctccctatcacat

SEQ ID NO: 127 - DNA, 41 bp, Artificial Sequence
  Synthetic sequence
gccctattgcaagccctcttgcctctagctagagagaagcg

SEQ ID NO: 128 - DNA, 39 bp, Artificial Sequence
  Synthetic sequence
gccctattgcaagccctcttctggcagtctagccattat

SEQ ID NO: 129 - DNA, 43 bp, Artificial Sequence
  Synthetic sequence
gccctattgcaagccctctttgtcttagaatttggcaactagt

SEQ ID NO: 130 - DNA, 39 bp, Artificial Sequence
  Synthetic sequence
gccctattgcaagccctcttgcaggaaagcctattgaat

SEQ ID NO: 131 - DNA, 39 bp, Artificial Sequence
  Synthetic sequence
gccctattgcaagccctcttgggagccagagaaatttct

SEQ ID NO: 132 - DNA, 44 bp, Artificial Sequence
  Synthetic sequence
gccctattgcaagccctctttgtctccagttccacttcatgtaa

SEQ ID NO: 133 - DNA, 39 bp, Artificial Sequence
  Synthetic sequence
gccctattgcaagccctcttcccgttaattgcctattta

SEQ ID NO: 134 - DNA, 38 bp, Artificial Sequence
  Synthetic sequence
gccctattgcaagccctcttctcggtcccactgggaaa

SEQ ID NO: 135 - DNA, 41 bp, Artificial Sequence
  Synthetic sequence
gccctattgcaagccctcttacacccatgattcagttacca

SEQ ID NO: 136 - DNA, 41 bp, Artificial Sequence
  Synthetic sequence
gccctattgcaagccctcttgctagtatgaacatcacaagt

SEQ ID NO: 137 - DNA, 43 bp, Artificial Sequence
  Synthetic sequence
gccctattgcaagccctcttacaaatgagtaagaagcgagtta

SEQ ID NO: 138 - DNA, 38 bp, Artificial Sequence
  Synthetic sequence
gccctattgcaagccctcttgataagggttgctctaca

SEQ ID NO: 139 - DNA, 37 bp, Artificial Sequence
  Synthetic sequence
gccctattgcaagccctcttccatgcaccagctacta

SEQ ID NO: 140 - DNA, 40 bp, Artificial Sequence
  Synthetic sequence
gccctattgcaagccctcttaactgtaccctactcccaat

SEQ ID NO: 141 - DNA, 41 bp, Artificial Sequence
  Synthetic sequence
gccctattgcaagccctcttaggaccaagggaccagttcac

SEQ ID NO: 142 - DNA, 42 bp, Artificial Sequence
  Synthetic sequence
gccctattgcaagccctcttagagttcctccaagaaattgta

SEQ ID NO: 143 - DNA, 44 bp, Artificial Sequence
  Synthetic sequence
gccctattgcaagccctcttacattatacagcatgctggttaga

SEQ ID NO: 144 - DNA, 41 bp, Artificial Sequence
  Synthetic sequence
gccctattgcaagccctcttgaggaagaaagtgagatttgt

SEQ ID NO: 145 - DNA, 44 bp, Artificial Sequence
  Synthetic sequence
gccctattgcaagccctcttctgaattatgtgcttaccaggagt

SEQ ID NO: 146 - DNA, 44 bp, Artificial Sequence
  Synthetic sequence
gccctattgcaagccctctttgggttctgataaccttatcaact

SEQ ID NO: 147 - DNA, 39 bp, Artificial Sequence
  Synthetic sequence
gccctattgcaagccctcttggttagtcaaacatgttgt

SEQ ID NO: 148 - DNA, 42 bp, Artificial Sequence
  Synthetic sequence
gccctattgcaagccctcttgacactggcagaatcaaaccaa

SEQ ID NO: 149 - DNA, 44 bp, Artificial Sequence
  Synthetic sequence
gccctattgcaagccctcttagagttacacctttagctaactag

SEQ ID NO: 150 - DNA, 38 bp, Artificial Sequence
  Synthetic sequence
gccctattgcaagccctcttccaggagttcaaggagca

SEQ ID NO: 151 - DNA, 41 bp, Artificial Sequence
  Synthetic sequence
gccctattgcaagccctcttaccactcctttctcccgtctt

SEQ ID NO: 152 - DNA, 44 bp, Artificial Sequence
  Synthetic sequence
gccctattgcaagccctcttgtcttatgggacaatggtcgatat

SEQ ID NO: 153 - DNA, 38 bp, Artificial Sequence
  Synthetic sequence
gccctattgcaagccctcttctaccctcaaccctcatt

SEQ ID NO: 154 - DNA, 38 bp, Artificial Sequence
  Synthetic sequence
gccctattgcaagccctcttccaagactgatcatgcta

SEQ ID NO: 155 - DNA, 61 bp, Artificial Sequence
  Synthetic sequence
cacttgacaaagttctcacgcgccgaagttctccgaaggatgccctcatcttcttccctgc

SEQ ID NO: 156 - DNA, 61 bp, Artificial Sequence
  Synthetic sequence
cattagggattaacggcttgggacagactgacggagcttcagccctcatcttcttccctgc

SEQ ID NO: 157 - DNA, 63 bp, Artificial Sequence
  Synthetic sequence
cacacgttaagaagactttctgctgactctgccgcacatgatcgccctcatcttcttccctgc

SEQ ID NO: 158 - DNA, 62 bp, Artificial Sequence
  Synthetic sequence
ctaagtgccctccatgagaaaggatccgatagccctctgcaggccctcatcttcttccctgc

SEQ ID NO: 159 - DNA, 60 bp, Artificial Sequence
  Synthetic sequence
gcacagatttcccacactctcaacaggcctgctaaacaccgccctcatcttcttccctgc

SEQ ID NO: 160 - DNA, 61 bp, Artificial Sequence
  Synthetic sequence
cttacaggaggtctggcatcaggtcaacaaccgagggactcgccctcatcttcttccctgc

SEQ ID NO: 161 - DNA, 59 bp, Artificial Sequence
  Synthetic sequence
ccacaatgagaaggcagagttgtcattaatgctggcggcgccctcatcttcttccctgc

SEQ ID NO: 162 - DNA, 60 bp, Artificial Sequence
  Synthetic sequence
gctgtggcatagctacactccggtgacggtttgcaactttgccctcatcttcttccctgc

SEQ ID NO: 163 - DNA, 60 bp, Artificial Sequence
  Synthetic sequence
cagggtaatttgtgggtctggtccggcagttaagggtctcgccctcatcttcttccctgc

SEQ ID NO: 164 - DNA, 62 bp, Artificial Sequence
  Synthetic sequence
gggctatccagaaagataagaatactcacaaacgactgcgcagccctcatcttcttccctgc

SEQ ID NO: 165 - DNA, 63 bp, Artificial Sequence
  Synthetic sequence
cataactggtggagtatttcactcgtatatggccgactggagggccctcatcttcttccctgc

SEQ ID NO: 166 - DNA, 64 bp, Artificial Sequence
  Synthetic sequence
cttcaaggaagaaattcaacagggtagggtttgcggcgataagggccctcatcttcttccctgc

SEQ ID NO: 167 - DNA, 62 bp, Artificial Sequence
  Synthetic sequence
catggattcaacacagcaaacaccaagtcaaccacccgagacgccctcatcttcttccctgc

SEQ ID NO: 168 - DNA, 62 bp, Artificial Sequence
  Synthetic sequence
ctctgacctccttcactcttacacttccctggccttccttctgccctcatcttcttccctgc

SEQ ID NO: 169 - DNA, 62 bp, Artificial Sequence
  Synthetic sequence
gctttcatttgtgctaaacctcgcttgggtcctctcctgaacgccctcatcttcttccctgc

SEQ ID NO: 170 - DNA, 58 bp, Artificial Sequence
  Synthetic sequence
catcccagatgccctcataacgtccgaaccacaatgctgccctcatcttcttccctgc

SEQ ID NO: 171 - DNA, 62 bp, Artificial Sequence
  Synthetic sequence
gtagaaatcccaaggcaatcagctcctcgcatccaacagtcggccctcatcttcttccctgc

SEQ ID NO: 172 - DNA, 63 bp, Artificial Sequence
  Synthetic sequence
gaacaactaactccacagaacccccaccgtagcactccttcttgccctcatcttcttccctgc

SEQ ID NO: 173 - DNA, 59 bp, Artificial Sequence
  Synthetic sequence
gtgcagaggacaggaagaacggagcgtcggtagtgtaaagccctcatcttcttccctgc

SEQ ID NO: 174 - DNA, 63 bp, Artificial Sequence
  Synthetic sequence
ggtgcttcaagacatacaccttaacaactcgacgaacctaccggccctcatcttcttccctgc

SEQ ID NO: 175 - DNA, 60 bp, Artificial Sequence
  Synthetic sequence
ggaacctctgtgaccttggatggcccatccttatgtgctggccctcatcttcttccctgc

SEQ ID NO: 176 - DNA, 59 bp, Artificial Sequence
  Synthetic sequence
cccagtggtaccttctgaaggtcgttattgctcaagcccgccctcatcttcttccctgc

SEQ ID NO: 177 - DNA, 63 bp, Artificial Sequence
  Synthetic sequence
cttctgttgcttatttgggtaacttgattctggccctcccatcgccctcatcttcttccctgc

SEQ ID NO: 178 - DNA, 56 bp, Artificial Sequence
  Synthetic sequence
cccactggatgcctccctcacgccggctatttaggtgccctcatcttcttccctgc

SEQ ID NO: 179 - DNA, 58 bp, Artificial Sequence
  Synthetic sequence
cggagagacgcatctgaaagtctgggtaggtggaggacgccctcatcttcttccctgc

SEQ ID NO: 180 - DNA, 61 bp, Artificial Sequence
  Synthetic sequence
caggatttccagcttacagggcgactgagccacatccaactgccctcatcttcttccctgc

SEQ ID NO: 181 - DNA, 60 bp, Artificial Sequence
  Synthetic sequence
cttgcaagatgtgcctcttagagcctcagccggaattgaagccctcatcttcttccctgc

SEQ ID NO: 182 - DNA, 62 bp, Artificial Sequence
  Synthetic sequence
gggtggtttctctaaacacaaattgccattctgcaccaatgcgccctcatcttcttccctgc

SEQ ID NO: 183 - DNA, 62 bp, Artificial Sequence
  Synthetic sequence
gcagggtattgagagaaggatctattggtgttcgcggctgatgccctcatcttcttccctgc

SEQ ID NO: 184 - DNA, 62 bp, Artificial Sequence
  Synthetic sequence
gtgcacatttcttgatgaagggatgggcgtaacaggaggactgccctcatcttcttccctgc

SEQ ID NO: 185 - DNA, 62 bp, Artificial Sequence
  Synthetic sequence
gagcaatgcctgtttcatgagaggaatggcctacctgcatcagccctcatcttcttccctgc

SEQ ID NO: 186 - DNA, 64 bp, Artificial Sequence
  Synthetic sequence
gttaacattatacagcatggtggccccgttgttgtcatcgcatcgccctcatcttcttccctgc

SEQ ID NO: 187 - DNA, 59 bp, Artificial Sequence
  Synthetic sequence
gcagaacatgtcctgaagcgttcgatgcgtcccatgagtgccctcatcttcttccctgc

SEQ ID NO: 188 - DNA, 60 bp, Artificial Sequence
  Synthetic sequence
cagcttgttcccaaacccatcaacccgcgtagatgttcctgccctcatcttcttccctgc

SEQ ID NO: 189 - DNA, 61 bp, Artificial Sequence
  Synthetic sequence
caaagtgtggaagttgcttccgccagctcaagagtgtagccgccctcatcttcttccctgc

SEQ ID NO: 190 - DNA, 58 bp, Artificial Sequence
  Synthetic sequence
ggtcgactttgtccatccttcttgatcctgcgcgatgtgccctcatcttcttccctgc

SEQ ID NO: 191 - DNA, 59 bp, Artificial Sequence
  Synthetic sequence
ctctgttgcctgtggactcatcgcaggcgttccctatacgccctcatcttcttccctgc

SEQ ID NO: 192 - DNA, 64 bp, Artificial Sequence
  Synthetic sequence
ctaactagaattagtctgcctgcctattggacctccgaccacgagccctcatcttcttccctgc

SEQ ID NO: 193 - DNA, 59 bp, Artificial Sequence
  Synthetic sequence
gtgagccataatcgtgtcaagccaccatttagatccgcggccctcatcttcttccctgc

SEQ ID NO: 194 - DNA, 63 bp, Artificial Sequence
  Synthetic sequence
gagaattaatgctccctctcctggaccagtagaagtctgcccggccctcatcttcttccctgc

SEQ ID NO: 195 - DNA, 59 bp, Artificial Sequence
  Synthetic sequence
gtggtctgctgttgaccaatttcagaatggccgagctgtgccctcatcttcttccctgc

SEQ ID NO: 196 - DNA, 60 bp, Artificial Sequence
  Synthetic sequence
ggttgcaactgctgatctataggtgaccttcttgtacgccgccctcatcttcttccctgc

SEQ ID NO: 197 - DNA, 58 bp, Artificial Sequence
  Synthetic sequence
ctttcccagtcaaggcagggcgcgtccttatttccatcgccctcatcttcttccctgc

SEQ ID NO: 198 - DNA, 20 bp, Artificial Sequence
  Synthetic sequence
agaccagcacaacttactcg

SEQ ID NO: 199 - DNA, 17 bp, Artificial Sequence
  Synthetic sequence
ccaaatgcacctgcctg

SEQ ID NO: 200 - DNA, 21 bp, Artificial Sequence
  Synthetic sequence
agtttggacaaaggcaattcg

SEQ ID NO: 201 - DNA, 24 bp, Artificial Sequence
  Synthetic sequence
tgagcttagccaatatcaagaagg

SEQ ID NO: 202 - DNA, 22 bp, Artificial Sequence
  Synthetic sequence
acgtgaactttccttggtacac

SEQ ID NO: 203 - DNA, 24 bp, Artificial Sequence
  Synthetic sequence
tgaagatgttctaataccttgccg

SEQ ID NO: 204 - DNA, 18 bp, Artificial Sequence
  Synthetic sequence
cagtgtggagactgaacg

SEQ ID NO: 205 - DNA, 23 bp, Artificial Sequence
  Synthetic sequence
aggcagggtaatgtcatgaaatg

SEQ ID NO: 206 - DNA, 17 bp, Artificial Sequence
  Synthetic sequence
gattgtctggagcgctg

SEQ ID NO: 207 - DNA, 16 bp, Artificial Sequence
  Synthetic sequence
agggagcaataggccg

SEQ ID NO: 208 - DNA, 17 bp, Artificial Sequence
  Synthetic sequence
ctgcagggtacaacacg

SEQ ID NO: 209 - DNA, 18 bp, Artificial Sequence
  Synthetic sequence
cgtatctgggaagacggc

SEQ ID NO: 210 - DNA, 20 bp, Artificial Sequence
  Synthetic sequence
cctgtaatcccttgcaatgc

SEQ ID NO: 211 - DNA, 18 bp, Artificial Sequence
  Synthetic sequence
ggtctcagcacggttctg

SEQ ID NO: 212 - DNA, 17 bp, Artificial Sequence
  Synthetic sequence
gcacctccctaccacac

SEQ ID NO: 213 - DNA, 21 bp, Artificial Sequence
  Synthetic sequence
gcctctagctagagagaagtc

SEQ ID NO: 214 - DNA, 19 bp, Artificial Sequence
  Synthetic sequence
ctggcagtctagccgttac

SEQ ID NO: 215 - DNA, 23 bp, Artificial Sequence
  Synthetic sequence
tgtcttagaatttggcaactggc

SEQ ID NO: 216 - DNA, 19 bp, Artificial Sequence
  Synthetic sequence
gcaggaaagcctactgaac

SEQ ID NO: 217 - DNA, 19 bp, Artificial Sequence
  Synthetic sequence
gggagccagagaaatgtcc

SEQ ID NO: 218 - DNA, 24 bp, Artificial Sequence
  Synthetic sequence
tgtctccagttccacttcatttag

SEQ ID NO: 219 - DNA, 19 bp, Artificial Sequence
  Synthetic sequence
cccgttaattgcctactcg

SEQ ID NO: 220 - DNA, 18 bp, Artificial Sequence
  Synthetic sequence
ctcggtcccactggaaag

SEQ ID NO: 221 - DNA, 21 bp, Artificial Sequence
  Synthetic sequence
acacccatgattcagttactg

SEQ ID NO: 222 - DNA, 21 bp, Artificial Sequence
  Synthetic sequence
gctagtatgaacatcacaggc

SEQ ID NO: 223 - DNA, 23 bp, Artificial Sequence
  Synthetic sequence
acaaatgagtaagaagcgagtcg

SEQ ID NO: 224 - DNA, 18 bp, Artificial Sequence
  Synthetic sequence
gataagggttgctctgcg

SEQ ID NO: 225 - DNA, 17 bp, Artificial Sequence
  Synthetic sequence
ccatgcaccagctaccc

SEQ ID NO: 226 - DNA, 20 bp, Artificial Sequence
  Synthetic sequence
aactgtaccctactcccagc

SEQ ID NO: 227 - DNA, 21 bp, Artificial Sequence
  Synthetic sequence
aggaccaagggaccagtttag

SEQ ID NO: 228 - DNA, 22 bp, Artificial Sequence
  Synthetic sequence
agagttcctccaagaaattgcg

SEQ ID NO: 229 - DNA, 24 bp, Artificial Sequence
  Synthetic sequence
acattatacagcatgctggctatc

SEQ ID NO: 230 - DNA, 21 bp, Artificial Sequence
  Synthetic sequence
gaggaagaaagtgaggtttgc

SEQ ID NO: 231 - DNA, 24 bp, Artificial Sequence
  Synthetic sequence
ctgaattatgtgcttaccaagagc

SEQ ID NO: 232 - DNA, 24 bp, Artificial Sequence
  Synthetic sequence
tgggttctgataaccttatcaagc

SEQ ID NO: 233 - DNA, 19 bp, Artificial Sequence
  Synthetic sequence
ggttagtcaaacatgctgc

SEQ ID NO: 234 - DNA, 22 bp, Artificial Sequence
  Synthetic sequence
gacactggcagaatcaaatcac

SEQ ID NO: 235 - DNA, 24 bp, Artificial Sequence
  Synthetic sequence
agagttacacctttagctaaccac

SEQ ID NO: 236 - DNA, 18 bp, Artificial Sequence
  Synthetic sequence
ccaggagttcaagaagcg

SEQ ID NO: 237 - DNA, 21 bp, Artificial Sequence
  Synthetic sequence
accactcctttctcccatctc

SEQ ID NO: 238 - DNA, 24 bp, Artificial Sequence
  Synthetic sequence
gtcttatgggacaatggttgatag

SEQ ID NO: 239 - DNA, 18 bp, Artificial Sequence
  Synthetic sequence
ctaccctcaaccctcgtc

SEQ ID NO: 240 - DNA, 18 bp, Artificial Sequence
  Synthetic sequence
ccaagactgatcatgccg

SEQ ID NO: 241 - DNA, 20 bp, Artificial Sequence
  Synthetic sequence
agaccagcacaacttactta

SEQ ID NO: 242 - DNA, 17 bp, Artificial Sequence
  Synthetic sequence
ccaaattcacctgccca

SEQ ID NO: 243 - DNA, 21 bp, Artificial Sequence
  Synthetic sequence
agtttggacaaaggcgattta

SEQ ID NO: 244 - DNA, 24 bp, Artificial Sequence
  Synthetic sequence
tgagcttagccaatatcaacaaga

SEQ ID NO: 245 - DNA, 22 bp, Artificial Sequence
  Synthetic sequence
acgtgaactttccttggtaaat

SEQ ID NO: 246 - DNA, 24 bp, Artificial Sequence
  Synthetic sequence
tgaagatgttctaataccttgcta

SEQ ID NO: 247 - DNA, 18 bp, Artificial Sequence
  Synthetic sequence
cagtgtggagaccgaaca

SEQ ID NO: 248 - DNA, 23 bp, Artificial Sequence
  Synthetic sequence
aggcagggtaatgtcatgaagtt

SEQ ID NO: 249 - DNA, 17 bp, Artificial Sequence
  Synthetic sequence
gattgtctggagggctc

SEQ ID NO: 250 - DNA, 16 bp, Artificial Sequence
  Synthetic sequence
agggagcaataggcta

SEQ ID NO: 251 - DNA, 17 bp, Artificial Sequence
  Synthetic sequence
ctgcagggtacaagaca

SEQ ID NO: 252 - DNA, 18 bp, Artificial Sequence
  Synthetic sequence
cgtatctgggaagatggg

SEQ ID NO: 253 - DNA, 20 bp, Artificial Sequence
  Synthetic sequence
cctgtaatcccttgcaataa

SEQ ID NO: 254 - DNA, 18 bp, Artificial Sequence
  Synthetic sequence
ggtctcagcacggtcctt

SEQ ID NO: 255 - DNA, 17 bp, Artificial Sequence
  Synthetic sequence
gcacctccctatcacat

SEQ ID NO: 256 - DNA, 21 bp, Artificial Sequence
  Synthetic sequence
gcctctagctagagagaagcg

SEQ ID NO: 257 - DNA, 19 bp, Artificial Sequence
  Synthetic sequence
ctggcagtctagccattat

SEQ ID NO: 258 - DNA, 23 bp, Artificial Sequence
  Synthetic sequence
tgtcttagaatttggcaactagt

SEQ ID NO: 259 - DNA, 19 bp, Artificial Sequence
  Synthetic sequence
gcaggaaagcctattgaat

SEQ ID NO: 260 - DNA, 19 bp, Artificial Sequence
  Synthetic sequence
gggagccagagaaatttct

SEQ ID NO: 261 - DNA, 24 bp, Artificial Sequence
  Synthetic sequence
tgtctccagttccacttcatgtaa

SEQ ID NO: 262 - DNA, 19 bp, Artificial Sequence
  Synthetic sequence
cccgttaattgcctattta

SEQ ID NO: 263 - DNA, 18 bp, Artificial Sequence
  Synthetic sequence
ctcggtcccactgggaaa

SEQ ID NO: 264 - DNA, 21 bp, Artificial Sequence
  Synthetic sequence
acacccatgattcagttacca

SEQ ID NO: 265 - DNA, 21 bp, Artificial Sequence
  Synthetic sequence
gctagtatgaacatcacaagt

SEQ ID NO: 266 - DNA, 23 bp, Artificial Sequence
  Synthetic sequence
acaaatgagtaagaagcgagtta

SEQ ID NO: 267 - DNA, 18 bp, Artificial Sequence
  Synthetic sequence
gataagggttgctctaca

SEQ ID NO: 268 - DNA, 17 bp, Artificial Sequence
  Synthetic sequence
ccatgcaccagctacta

SEQ ID NO: 269 - DNA, 20 bp, Artificial Sequence
  Synthetic sequence
aactgtaccctactcccaat

SEQ ID NO: 270 - DNA, 21 bp, Artificial Sequence
  Synthetic sequence
aggaccaagggaccagttcac

SEQ ID NO: 271 - DNA, 22 bp, Artificial Sequence
  Synthetic sequence
agagttcctccaagaaattgta

SEQ ID NO: 272 - DNA, 24 bp, Artificial Sequence
  Synthetic sequence
acattatacagcatgctggttaga

SEQ ID NO: 273 - DNA, 21 bp, Artificial Sequence
  Synthetic sequence
gaggaagaaagtgagatttgt

SEQ ID NO: 274 - DNA, 24 bp, Artificial Sequence
  Synthetic sequence
ctgaattatgtgcttaccaggagt

SEQ ID NO: 275 - DNA, 24 bp, Artificial Sequence
  Synthetic sequence
tgggttctgataaccttatcaact

SEQ ID NO: 276 - DNA, 19 bp, Artificial Sequence
  Synthetic sequence
ggttagtcaaacatgttgt

SEQ ID NO: 277 - DNA, 22 bp, Artificial Sequence
  Synthetic sequence
gacactggcagaatcaaaccaa

SEQ ID NO: 278 - DNA, 24 bp, Artificial Sequence
  Synthetic sequence
agagttacacctttagctaactag

SEQ ID NO: 279 - DNA, 18 bp, Artificial Sequence
  Synthetic sequence
ccaggagttcaaggagca

SEQ ID NO: 280 - DNA, 21 bp, Artificial Sequence
  Synthetic sequence
accactcctttctcccgtctt

SEQ ID NO: 281 - DNA, 24 bp, Artificial Sequence
  Synthetic sequence
gtcttatgggacaatggtcgatat

SEQ ID NO: 282 - DNA, 18 bp, Artificial Sequence
  Synthetic sequence
ctaccctcaaccctcatt

SEQ ID NO: 283 - DNA, 18 bp, Artificial Sequence
  Synthetic sequence
ccaagactgatcatgcta

SEQ ID NO: 284 - DNA, 21 bp, Artificial Sequence
  Synthetic sequence
cacttgacaaagttctcacgc

SEQ ID NO: 285 - DNA, 21 bp, Artificial Sequence
  Synthetic sequence
cattagggattaacggcttgg

SEQ ID NO: 286 - DNA, 23 bp, Artificial Sequence
  Synthetic sequence
cacacgttaagaagactttctgc

SEQ ID NO: 287 - DNA, 22 bp, Artificial Sequence
  Synthetic sequence
ctaagtgccctccatgagaaag

SEQ ID NO: 288 - DNA, 20 bp, Artificial Sequence
  Synthetic sequence
gcacagatttcccacactct

SEQ ID NO: 289 - DNA, 21 bp, Artificial Sequence
  Synthetic sequence
cttacaggaggtctggcatca

SEQ ID NO: 290 - DNA, 19 bp, Artificial Sequence
  Synthetic sequence
ccacaatgagaaggcagag

SEQ ID NO: 291 - DNA, 20 bp, Artificial Sequence
  Synthetic sequence
gctgtggcatagctacactc

SEQ ID NO: 292 - DNA, 20 bp, Artificial Sequence
  Synthetic sequence
cagggtaatttgtgggtctg

SEQ ID NO: 293 - DNA, 22 bp, Artificial Sequence
  Synthetic sequence
gggctatccagaaagataagaa

SEQ ID NO: 294 - DNA, 23 bp, Artificial Sequence
  Synthetic sequence
cataactggtggagtatttcact

SEQ ID NO: 295 - DNA, 24 bp, Artificial Sequence
  Synthetic sequence
cttcaaggaagaaattcaacaggg

SEQ ID NO: 296 - DNA, 22 bp, Artificial Sequence
  Synthetic sequence
catggattcaacacagcaaaca

SEQ ID NO: 297 - DNA, 22 bp, Artificial Sequence
  Synthetic sequence
ctctgacctccttcactcttac

SEQ ID NO: 298 - DNA, 22 bp, Artificial Sequence
  Synthetic sequence
gctttcatttgtgctaaacctc

SEQ ID NO: 299 - DNA, 18 bp, Artificial Sequence
  Synthetic sequence
catcccagatgccctcat

SEQ ID NO: 300 - DNA, 22 bp, Artificial Sequence
  Synthetic sequence
gtagaaatcccaaggcaatcag

SEQ ID NO: 301 - DNA, 23 bp, Artificial Sequence
  Synthetic sequence
gaacaactaactccacagaaccc

SEQ ID NO: 302 - DNA, 19 bp, Artificial Sequence
  Synthetic sequence
gtgcagaggacaggaagaa

SEQ ID NO: 303 - DNA, 23 bp, Artificial Sequence
  Synthetic sequence
ggtgcttcaagacatacacctta

SEQ ID NO: 304 - DNA, 20 bp, Artificial Sequence
  Synthetic sequence
ggaacctctgtgaccttgga

SEQ ID NO: 305 - DNA, 19 bp, Artificial Sequence
  Synthetic sequence
cccagtggtaccttctgaa

SEQ ID NO: 306 - DNA, 23 bp, Artificial Sequence
  Synthetic sequence
cttctgttgcttatttgggtaac

SEQ ID NO: 307 - DNA, 16 bp, Artificial Sequence
  Synthetic sequence
cccactggatgcctcc

SEQ ID NO: 308 - DNA, 18 bp, Artificial Sequence
  Synthetic sequence
cggagagacgcatctgaa

SEQ ID NO: 309 - DNA, 21 bp, Artificial Sequence
  Synthetic sequence
caggatttccagcttacaggg

SEQ ID NO: 310 - DNA, 20 bp, Artificial Sequence
  Synthetic sequence
cttgcaagatgtgcctctta

SEQ ID NO: 311 - DNA, 22 bp, Artificial Sequence
  Synthetic sequence
gggtggtttctctaaacacaaa

SEQ ID NO: 312 - DNA, 22 bp, Artificial Sequence
  Synthetic sequence
gcagggtattgagagaaggatc

SEQ ID NO: 313 - DNA, 22 bp, Artificial Sequence
  Synthetic sequence
gtgcacatttcttgatgaaggg

SEQ ID NO: 314 - DNA, 22 bp, Artificial Sequence
  Synthetic sequence
gagcaatgcctgtttcatgaga

SEQ ID NO: 315 - DNA, 24 bp, Artificial Sequence
  Synthetic sequence
gttaacattatacagcatggtggc

SEQ ID NO: 316 - DNA, 19 bp, Artificial Sequence
  Synthetic sequence
gcagaacatgtcctgaagc

SEQ ID NO: 317 - DNA, 20 bp, Artificial Sequence
  Synthetic sequence
cagcttgttcccaaacccat

SEQ ID NO: 318 - DNA, 21 bp, Artificial Sequence
  Synthetic sequence
caaagtgtggaagttgcttcc

SEQ ID NO: 319 - DNA, 18 bp, Artificial Sequence
  Synthetic sequence
ggtcgactttgtccatcc

SEQ ID NO: 320 - DNA, 19 bp, Artificial Sequence
  Synthetic sequence
ctctgttgcctgtggactc

SEQ ID NO: 321 - DNA, 24 bp, Artificial Sequence
  Synthetic sequence
ctaactagaattagtctgcctgcc

SEQ ID NO: 322 - DNA, 19 bp, Artificial Sequence
  Synthetic sequence
gtgagccataatcgtgtca

SEQ ID NO: 323 - DNA, 23 bp, Artificial Sequence
  Synthetic sequence
gagaattaatgctccctctcctg

SEQ ID NO: 324 - DNA, 19 bp, Artificial Sequence
  Synthetic sequence
gtggtctgctgttgaccaa

SEQ ID NO: 325 - DNA, 20 bp, Artificial Sequence
  Synthetic sequence
ggttgcaactgctgatctat

SEQ ID NO: 326 - DNA, 18 bp, Artificial Sequence
  Synthetic sequence
ctttcccagtcaaggcag

SEQ ID NO: 327 - DNA, 20 bp, Artificial Sequence
  Synthetic sequence
gccgaagttctccgaaggat

SEQ ID NO: 328 - DNA, 20 bp, Artificial Sequence
  Synthetic sequence
gacagactgacggagcttca

SEQ ID NO: 329 - DNA, 20 bp, Artificial Sequence
  Synthetic sequence
tgactctgccgcacatgatc

SEQ ID NO: 330 - DNA, 20 bp, Artificial Sequence
  Synthetic sequence
gatccgatagccctctgcag

SEQ ID NO: 331 - DNA, 20 bp, Artificial Sequence
  Synthetic sequence
caacaggcctgctaaacacc

SEQ ID NO: 332 - DNA, 20 bp, Artificial Sequence
  Synthetic sequence
ggtcaacaaccgagggactc

SEQ ID NO: 333 - DNA, 20 bp, Artificial Sequence
  Synthetic sequence
ttgtcattaatgctggcggc

SEQ ID NO: 334 - DNA, 20 bp, Artificial Sequence
  Synthetic sequence
cggtgacggtttgcaacttt

SEQ ID NO: 335 - DNA, 20 bp, Artificial Sequence
  Synthetic sequence
gtccggcagttaagggtctc

SEQ ID NO: 336 - DNA, 20 bp, Artificial Sequence
  Synthetic sequence
tactcacaaacgactgcgca

SEQ ID NO: 337 - DNA, 20 bp, Artificial Sequence
  Synthetic sequence
cgtatatggccgactggagg

SEQ ID NO: 338 - DNA, 20 bp, Artificial Sequence
  Synthetic sequence
tagggtttgcggcgataagg

SEQ ID NO: 339 - DNA, 20 bp, Artificial Sequence
  Synthetic sequence
ccaagtcaaccacccgagac

SEQ ID NO: 340 - DNA, 20 bp, Artificial Sequence
  Synthetic sequence
acttccctggccttccttct

SEQ ID NO: 341 - DNA, 20 bp, Artificial Sequence
  Synthetic sequence
gcttgggtcctctcctgaac

SEQ ID NO: 342 - DNA, 20 bp, Artificial Sequence
  Synthetic sequence
aacgtccgaaccacaatgct

SEQ ID NO: 343 - DNA, 20 bp, Artificial Sequence
  Synthetic sequence
ctcctcgcatccaacagtcg

SEQ ID NO: 344 - DNA, 20 bp, Artificial Sequence
  Synthetic sequence
ccaccgtagcactccttctt

SEQ ID NO: 345 - DNA, 20 bp, Artificial Sequence
  Synthetic sequence
cggagcgtcggtagtgtaaa

SEQ ID NO: 346 - DNA, 20 bp, Artificial Sequence
  Synthetic sequence
acaactcgacgaacctaccg

SEQ ID NO: 347 - DNA, 20 bp, Artificial Sequence
  Synthetic sequence
tggcccatccttatgtgctg

SEQ ID NO: 348 - DNA, 20 bp, Artificial Sequence
  Synthetic sequence
ggtcgttattgctcaagccc

SEQ ID NO: 349 - DNA, 20 bp, Artificial Sequence
  Synthetic sequence
ttgattctggccctcccatc

SEQ ID NO: 350 - DNA, 20 bp, Artificial Sequence
  Synthetic sequence
ctcacgccggctatttaggt

SEQ ID NO: 351 - DNA, 20 bp, Artificial Sequence
  Synthetic sequence
agtctgggtaggtggaggac

SEQ ID NO: 352 - DNA, 20 bp, Artificial Sequence
  Synthetic sequence
cgactgagccacatccaact

SEQ ID NO: 353 - DNA, 20 bp, Artificial Sequence
  Synthetic sequence
gagcctcagccggaattgaa

SEQ ID NO: 354 - DNA, 20 bp, Artificial Sequence
  Synthetic sequence
ttgccattctgcaccaatgc

SEQ ID NO: 355 - DNA, 20 bp, Artificial Sequence
  Synthetic sequence
tattggtgttcgcggctgat

SEQ ID NO: 356 - DNA, 20 bp, Artificial Sequence
  Synthetic sequence
atgggcgtaacaggaggact

SEQ ID NO: 357 - DNA, 20 bp, Artificial Sequence
  Synthetic sequence
ggaatggcctacctgcatca

SEQ ID NO: 358 - DNA, 20 bp, Artificial Sequence
  Synthetic sequence
cccgttgttgtcatcgcatc

SEQ ID NO: 359 - DNA, 20 bp, Artificial Sequence
  Synthetic sequence
gttcgatgcgtcccatgagt

SEQ ID NO: 360 - DNA, 20 bp, Artificial Sequence
  Synthetic sequence
caacccgcgtagatgttcct

SEQ ID NO: 361 - DNA, 20 bp, Artificial Sequence
  Synthetic sequence
gccagctcaagagtgtagcc

SEQ ID NO: 362 - DNA, 20 bp, Artificial Sequence
  Synthetic sequence
ttcttgatcctgcgcgatgt

SEQ ID NO: 363 - DNA, 20 bp, Artificial Sequence
  Synthetic sequence
atcgcaggcgttccctatac

SEQ ID NO: 364 - DNA, 20 bp, Artificial Sequence
  Synthetic sequence
tattggacctccgaccacga

SEQ ID NO: 365 - DNA, 20 bp, Artificial Sequence
  Synthetic sequence
agccaccatttagatccgcg

SEQ ID NO: 366 - DNA, 20 bp, Artificial Sequence
  Synthetic sequence
gaccagtagaagtctgcccg

SEQ ID NO: 367 - DNA, 20 bp, Artificial Sequence
  Synthetic sequence
tttcagaatggccgagctgt

SEQ ID NO: 368 - DNA, 20 bp, Artificial Sequence
  Synthetic sequence
aggtgaccttcttgtacgcc

SEQ ID NO: 369 - DNA, 20 bp, Artificial Sequence
  Synthetic sequence
ggcgcgtccttatttccatc